European Patent Application EP 4 276 107 A2, published November 15, 2023. Title: GlxR protein variant or threonine production method using the same. Applicant: CJ CheilJedang Corporation. The sequence listing filed with the application follows.

SEQUENCE LISTING (55 sequences)

SEQ ID NO: 1 - protein, 227 aa, Artificial Sequence
  GlxR_amino acid
MEGVQEILSRAGIFQGVDPTAVNNLIQDMETVRFPRGATIFDEGEPGDRLYIITSGKVKLARHAPDGRENLLTIMGPSDMFGELSIFDPGPRTSSAVCVTEVHAATMNSDMLRNWVADHPAIAEQLLRVLARRLRRTNASLADLIFTDVPGRVAKTLLQLANRFGTQEAGALRVNHDLTQEEIAQLVGASRETVNKALATFAHRGWIRLEGKSVLIVDTEHLARRAR

SEQ ID NO: 2 - DNA, 684 bp, Artificial Sequence
  glxR_nucleic acid
gtggaaggtgtacaggagatcctgtcgcgcgccggaatttttcaaggcgttgacccaacggcagtcaataacctcatccaggatatggagaccgttcgcttcccacgcggagcaaccatcttcgacgagggcgagccaggtgaccgcctttacatcatcacctccggcaaagtgaagcttgcgcgccacgcaccggacggccgcgaaaacctgctgaccatcatgggtccttccgacatgttcggtgagctctccatcttcgacccaggcccacgcacctcctctgcagtgtgtgtcaccgaagttcatgcagcaaccatgaactctgacatgctgcgcaactgggtagctgaccacccagctatcgctgagcagctcctgcgcgttctggctcgtcgtctgcgtcgcaccaacgcttccctggctgacctcatcttcaccgacgtcccaggccgcgttgctaagacccttctgcagctggctaaccgcttcggcacccaagaagctggcgcgctgcgcgtgaaccacgacctcactcaggaagaaatcgcacagctcgtcggtgcttcccgtgaaactgtgaataaggctcttgcaacgttcgcacaccgtggctggattcgcctcgagggcaagtccgtcctcattgtggacaccgagcatttggcacgtcgcgctcgataa

SEQ ID NO: 3 - protein, 227 aa, Artificial Sequence
  GlxR_E45A
MEGVQEILSRAGIFQGVDPTAVNNLIQDMETVRFPRGATIFDEGAPGDRLYIITSGKVKLARHAPDGRENLLTIMGPSDMFGELSIFDPGPRTSSAVCVTEVHAATMNSDMLRNWVADHPAIAEQLLRVLARRLRRTNASLADLIFTDVPGRVAKTLLQLANRFGTQEAGALRVNHDLTQEEIAQLVGASRETVNKALATFAHRGWIRLEGKSVLIVDTEHLARRAR

SEQ ID NO: 4 - protein, 227 aa, Artificial Sequence
  GlxR_E45S
MEGVQEILSRAGIFQGVDPTAVNNLIQDMETVRFPRGATIFDEGSPGDRLYIITSGKVKLARHAPDGRENLLTIMGPSDMFGELSIFDPGPRTSSAVCVTEVHAATMNSDMLRNWVADHPAIAEQLLRVLARRLRRTNASLADLIFTDVPGRVAKTLLQLANRFGTQEAGALRVNHDLTQEEIAQLVGASRETVNKALATFAHRGWIRLEGKSVLIVDTEHLARRAR

SEQ ID NO: 5 - protein, 227 aa, Artificial Sequence
  GlxR_E45F
MEGVQEILSRAGIFQGVDPTAVNNLIQDMETVRFPRGATIFDEGFPGDRLYIITSGKVKLARHAPDGRENLLTIMGPSDMFGELSIFDPGPRTSSAVCVTEVHAATMNSDMLRNWVADHPAIAEQLLRVLARRLRRTNASLADLIFTDVPGRVAKTLLQLANRFGTQEAGALRVNHDLTQEEIAQLVGASRETVNKALATFAHRGWIRLEGKSVLIVDTEHLARRAR

SEQ ID NO: 6 - protein, 227 aa, Artificial Sequence
  GlxR_E45K
MEGVQEILSRAGIFQGVDPTAVNNLIQDMETVRFPRGATIFDEGKPGDRLYIITSGKVKLARHAPDGRENLLTIMGPSDMFGELSIFDPGPRTSSAVCVTEVHAATMNSDMLRNWVADHPAIAEQLLRVLARRLRRTNASLADLIFTDVPGRVAKTLLQLANRFGTQEAGALRVNHDLTQEEIAQLVGASRETVNKALATFAHRGWIRLEGKSVLIVDTEHLARRAR

SEQ ID NO: 7 - protein, 227 aa, Artificial Sequence
  GlxR_D66A
MEGVQEILSRAGIFQGVDPTAVNNLIQDMETVRFPRGATIFDEGEPGDRLYIITSGKVKLARHAPAGRENLLTIMGPSDMFGELSIFDPGPRTSSAVCVTEVHAATMNSDMLRNWVADHPAIAEQLLRVLARRLRRTNASLADLIFTDVPGRVAKTLLQLANRFGTQEAGALRVNHDLTQEEIAQLVGASRETVNKALATFAHRGWIRLEGKSVLIVDTEHLARRAR

SEQ ID NO: 8 - protein, 227 aa, Artificial Sequence
  GlxR_D66F
MEGVQEILSRAGIFQGVDPTAVNNLIQDMETVRFPRGATIFDEGEPGDRLYIITSGKVKLARHAPFGRENLLTIMGPSDMFGELSIFDPGPRTSSAVCVTEVHAATMNSDMLRNWVADHPAIAEQLLRVLARRLRRTNASLADLIFTDVPGRVAKTLLQLANRFGTQEAGALRVNHDLTQEEIAQLVGASRETVNKALATFAHRGWIRLEGKSVLIVDTEHLARRAR

SEQ ID NO: 9 - protein, 227 aa, Artificial Sequence
  GlxR_D66K
MEGVQEILSRAGIFQGVDPTAVNNLIQDMETVRFPRGATIFDEGEPGDRLYIITSGKVKLARHAPKGRENLLTIMGPSDMFGELSIFDPGPRTSSAVCVTEVHAATMNSDMLRNWVADHPAIAEQLLRVLARRLRRTNASLADLIFTDVPGRVAKTLLQLANRFGTQEAGALRVNHDLTQEEIAQLVGASRETVNKALATFAHRGWIRLEGKSVLIVDTEHLARRAR

SEQ ID NO: 10 - protein, 227 aa, Artificial Sequence
  GlxR_T166D
MEGVQEILSRAGIFQGVDPTAVNNLIQDMETVRFPRGATIFDEGEPGDRLYIITSGKVKLARHAPDGRENLLTIMGPSDMFGELSIFDPGPRTSSAVCVTEVHAATMNSDMLRNWVADHPAIAEQLLRVLARRLRRTNASLADLIFTDVPGRVAKTLLQLANRFGDQEAGALRVNHDLTQEEIAQLVGASRETVNKALATFAHRGWIRLEGKSVLIVDTEHLARRAR

SEQ ID NO: 11 - protein, 227 aa, Artificial Sequence
  GlxR_T166F
MEGVQEILSRAGIFQGVDPTAVNNLIQDMETVRFPRGATIFDEGEPGDRLYIITSGKVKLARHAPDGRENLLTIMGPSDMFGELSIFDPGPRTSSAVCVTEVHAATMNSDMLRNWVADHPAIAEQLLRVLARRLRRTNASLADLIFTDVPGRVAKTLLQLANRFGFQEAGALRVNHDLTQEEIAQLVGASRETVNKALATFAHRGWIRLEGKSVLIVDTEHLARRAR

SEQ ID NO: 12 - protein, 227 aa, Artificial Sequence
  GlxR_T166K
MEGVQEILSRAGIFQGVDPTAVNNLIQDMETVRFPRGATIFDEGEPGDRLYIITSGKVKLARHAPDGRENLLTIMGPSDMFGELSIFDPGPRTSSAVCVTEVHAATMNSDMLRNWVADHPAIAEQLLRVLARRLRRTNASLADLIFTDVPGRVAKTLLQLANRFGKQEAGALRVNHDLTQEEIAQLVGASRETVNKALATFAHRGWIRLEGKSVLIVDTEHLARRAR

SEQ ID NO: 13 - protein, 227 aa, Artificial Sequence
  GlxR_E168A
MEGVQEILSRAGIFQGVDPTAVNNLIQDMETVRFPRGATIFDEGEPGDRLYIITSGKVKLARHAPDGRENLLTIMGPSDMFGELSIFDPGPRTSSAVCVTEVHAATMNSDMLRNWVADHPAIAEQLLRVLARRLRRTNASLADLIFTDVPGRVAKTLLQLANRFGTQAAGALRVNHDLTQEEIAQLVGASRETVNKALATFAHRGWIRLEGKSVLIVDTEHLARRAR

SEQ ID NO: 14 - protein, 227 aa, Artificial Sequence
  GlxR_E168F
MEGVQEILSRAGIFQGVDPTAVNNLIQDMETVRFPRGATIFDEGEPGDRLYIITSGKVKLARHAPDGRENLLTIMGPSDMFGELSIFDPGPRTSSAVCVTEVHAATMNSDMLRNWVADHPAIAEQLLRVLARRLRRTNASLADLIFTDVPGRVAKTLLQLANRFGTQFAGALRVNHDLTQEEIAQLVGASRETVNKALATFAHRGWIRLEGKSVLIVDTEHLARRAR

SEQ ID NO: 15 - protein, 227 aa, Artificial Sequence
  GlxR_E168K
MEGVQEILSRAGIFQGVDPTAVNNLIQDMETVRFPRGATIFDEGEPGDRLYIITSGKVKLARHAPDGRENLLTIMGPSDMFGELSIFDPGPRTSSAVCVTEVHAATMNSDMLRNWVADHPAIAEQLLRVLARRLRRTNASLADLIFTDVPGRVAKTLLQLANRFGTQKAGALRVNHDLTQEEIAQLVGASRETVNKALATFAHRGWIRLEGKSVLIVDTEHLARRAR

SEQ ID NO: 16 - DNA, 35 bp, Artificial Sequence
  glxR L1
gaattcgagctcggtaccctgagaccccacgcgag

SEQ ID NO: 17 - DNA, 36 bp, Artificial Sequence
  glxR R2
gactctagaggatccccatcgacggtgtcaccccac

SEQ ID NO: 18 - DNA, 38 bp, Artificial Sequence
  glxR(E45A) L2
gtaaaggcggtcacctggcgcgccctcgtcgaagatgg

SEQ ID NO: 19 - DNA, 38 bp, Artificial Sequence
  glxR(E45A) R1
ccatcttcgacgagggcgcgccaggtgaccgcctttac

SEQ ID NO: 20 - DNA, 21 bp, Artificial Sequence
  pDZ_F (pDZ vector sequencing primer_forward)
tattacgccagctggcgaaag

SEQ ID NO: 21 - DNA, 21 bp, Artificial Sequence
  pDZ_R (pDZ vector sequencing primer_reverse)
ttccggctcgtatgttgtgtg

SEQ ID NO: 22 - DNA, 38 bp, Artificial Sequence
  glxR(E45S) L2
gtaaaggcggtcacctggagagccctcgtcgaagatgg

SEQ ID NO: 23 - DNA, 38 bp, Artificial Sequence
  glxR(E45S) R1
ccatcttcgacgagggctctccaggtgaccgcctttac

SEQ ID NO: 24 - DNA, 38 bp, Artificial Sequence
  glxR(E45F) L2
gtaaaggcggtcacctggaaagccctcgtcgaagatgg

SEQ ID NO: 25 - DNA, 38 bp, Artificial Sequence
  glxR(E45F) R1
ccatcttcgacgagggctttccaggtgaccgcctttac

SEQ ID NO: 26 - DNA, 38 bp, Artificial Sequence
  glxR(E45K) L2
gtaaaggcggtcacctggcttgccctcgtcgaagatgg

SEQ ID NO: 27 - DNA, 38 bp, Artificial Sequence
  glxR(E45K) R1
ccatcttcgacgagggcaagccaggtgaccgcctttac

SEQ ID NO: 28 - DNA, 34 bp, Artificial Sequence
  glxR(D66A) L2
ggttttcgcggcctgccggtgcgtggcgcgcaag

SEQ ID NO: 29 - DNA, 34 bp, Artificial Sequence
  glxR(D66A) R1
gcgccacgcaccggcaggccgcgaaaacctgctg

SEQ ID NO: 30 - DNA, 34 bp, Artificial Sequence
  glxR(D66F) L2
cagcaggttttcgcggccaaacggtgcgtggcgc

SEQ ID NO: 31 - DNA, 34 bp, Artificial Sequence
  glxR(D66F) R1
gcgccacgcaccgtttggccgcgaaaacctgctg

SEQ ID NO: 32 - DNA, 35 bp, Artificial Sequence
  glxR(D66K) L2
ggttttcgcggcctttccggtgcgtggcgcgcaag

SEQ ID NO: 33 - DNA, 34 bp, Artificial Sequence
  glxR(D66K) R1
gcgccacgcaccgaaaggccgcgaaaacctgctg

SEQ ID NO: 34 - DNA, 34 bp, Artificial Sequence
  glxR(T166D) L2
gccagcttcttggtcgccgaagcggttagccagc

SEQ ID NO: 35 - DNA, 33 bp, Artificial Sequence
  glxR(T166D) R1
aaccgcttcggcgaccaagaagctggcgcgctg

SEQ ID NO: 36 - DNA, 34 bp, Artificial Sequence
  glxR(T166F) L2
gccagcttcttggaagccgaagcggttagccagc

SEQ ID NO: 37 - DNA, 33 bp, Artificial Sequence
  glxR(T166F) R1
aaccgcttcggcttccaagaagctggcgcgctg

SEQ ID NO: 38 - DNA, 34 bp, Artificial Sequence
  glxR(T166K) L2
gccagcttcttgtttgccgaagcggttagccagc

SEQ ID NO: 39 - DNA, 33 bp, Artificial Sequence
  glxR(T166K) R1
aaccgcttcggcaaacaagaagctggcgcgctg

SEQ ID NO: 40 - DNA, 34 bp, Artificial Sequence
  glxR(E168A) L2
agcgcgccagcagcttgggcgccgaagcggttag

SEQ ID NO: 41 - DNA, 34 bp, Artificial Sequence
  glxR(E168A) R1
cttcggcgcccaagctgctggcgcgctgcgcgtg

SEQ ID NO: 42 - DNA, 34 bp, Artificial Sequence
  glxR(E168F) L2
agcgcgccagcaaattgggcgccgaagcggttag

SEQ ID NO: 43 - DNA, 34 bp, Artificial Sequence
  glxR(E168F) R1
cttcggcgcccaatttgctggcgcgctgcgcgtg

SEQ ID NO: 44 - DNA, 34 bp, Artificial Sequence
  glxR(E168K) L2
agcgcgccagccttttgggcgccgaagcggttag

SEQ ID NO: 45 - DNA, 34 bp, Artificial Sequence
  glxR(E168K) R1
cttcggcgcccaaaaggctggcgcgctgcgcgtg

SEQ ID NO: 46 - protein, 421 aa, Artificial Sequence
  LysC_L377K
MALVVQKYGGSSLESAERIRNVAERIVATKKAGNDVVVVCSAMGDTTDELLELAAAVNPVPPAREMDMLLTAGERISNALVAMAIESLGAEAQSFTGSQAGVLTTERHGNARIVDVTPGRVREALDEGKICIVAGFQGVNKETRDVTTLGRGGSDTTAVALAAALNADVCEIYSDVDGVYTADPRIVPNAQKLEKLSFEEMLELAAVGSKILVLRSVEYARAFNVPLRVRSSYSNDPGTLIAGSMEDIPVEEAVLTGVATDKSEAKVTVLGISDKPGEAAKVFRALADAEINIDMVLQNVSSVEDGTTDITFTCPRSDGRRAMEILKKLQVQGNWTNVLYDDQVGKVSLVGAGMKSHPGVTAEFMEALRDVNVNIEKISTSEIRISVLIREDDLDAAARALHEQFQLGGEDEAVVYAGTGR

SEQ ID NO: 47 - DNA, 34 bp, Artificial Sequence
  lysC L1
tcgagctcggtacccgctgcgcagtgttgaatac

SEQ ID NO: 48 - DNA, 34 bp, Artificial Sequence
  lysC R2
ctctagaggatccccgttcacctcagagacgatt

SEQ ID NO: 49 - DNA, 30 bp, Artificial Sequence
  lysC(L377K) L2
tggaaatcttttcgatgttcacgttgacat

SEQ ID NO: 50 - DNA, 30 bp, Artificial Sequence
  lysC(L377K) R1
atgtcaacgtgaacatcgaaaagatttcca

SEQ ID NO: 51 - protein, 445 aa, Artificial Sequence
  Hom_R407H
MTSASAPSFNPGKGPGSAVGIALLGFGTVGTEVMRLMTEYGDELAHRIGGPLEVRGIAVSDISKPREGVAPELLTEDAFALIEREDVDIVVEVIGGIEYPREVVLAALKAGKSVVTANKALVAAHSAELADAAEAANVDLYFEAAVAGAIPVVGPLRRSLAGDQIQSVMGIVNGTTNFILDAMDSTGADYADSLAEATRLGYAEADPTADVEGHDAASKAAILASIAFHTRVTADDVYCEGISNISAADIEAAQQAGHTIKLLAICEKFTNKEGKSAISARVHPTLLPVSHPLASVNKSFNAIFVEAEAAGRLMFYGNGAGGAPTASAVLGDVVGAARNKVHGGRAPGESTYANLPIADFGETTTRYHLDMDVEDRVGVLAELASLFSEQGISLRTIRQEERDDDAHLIVVTHSALESDLSRTVELLKAKPVVKAINSVIRLERD

SEQ ID NO: 52 - DNA, 34 bp, Artificial Sequence
  hom L1
atcctctagagtcgacccaactgcagacgtcgaa

SEQ ID NO: 53 - DNA, 35 bp, Artificial Sequence
  hom R2
atgcctgcaggtcgacatagacagatttgtccacg

SEQ ID NO: 54 - DNA, 35 bp, Artificial Sequence
  hom(R407H) L2
gtgaccacgatcagatgtgcatcatcatcgcgctc

SEQ ID NO: 55 - DNA, 35 bp, Artificial Sequence
  hom(R407H) R1
gcgatgatgatgcacatctgatcgtggtcacccac